European Patent Application EP 4 403 645 A1, published July 24, 2024. Title: DETECTION OF TARGET NUCLEIC ACID SEQUENCE USING TAG OLIGONUCLEOTIDE COMPRISING SYNTHETIC UNNATURAL BASE. Applicant: SEEGENE, INC. The sequence listing filed with the application follows.

SEQUENCE LISTING (17 sequences)

SEQ ID NO: 1 - DNA, 215 bp, Enterococcus faecalis
  source 1..215: mol_type = other DNA
ccacaagtaccattcgtgccagttttaagaagtgactggaaaggaaatccaaaagaagtctttgaaaaatgtgaaggttctttaatttatccggtctttgttaaacctgccaatatgggttctagtgtcggaattagcaaagcggaaaatcgtgaagaattgcaagaagcattggaagaagctttccgttatgatgcccgagcaattgttgaaca

SEQ ID NO: 2 - DNA, 20 bp, synthetic construct
  source 1..20: mol_type = other DNA
ccacaagtaccattcgtgcc

SEQ ID NO: 3 - DNA, 20 bp, synthetic construct
  source 1..20: mol_type = other DNA
tgttcaacaattgctcgrgc

SEQ ID NO: 4 - DNA, 38 bp, synthetic construct
  source 1..38: mol_type = other DNA
  misc_feature 12: note = n is unnatural base, P
cgcattctcgtncgtgaagaattgcaagaagcattgga

SEQ ID NO: 5 - DNA, 38 bp, synthetic construct
  source 1..38: mol_type = other DNA
  misc_feature 27: note = n is unnatural base, Z
acgtcgattcgccgcgtcgatagacgnacgagaatgcg

SEQ ID NO: 6 - DNA, 38 bp, synthetic construct
  source 1..38: mol_type = other DNA
  misc_feature 11: note = n is unnatural base, P
cgcattctcgnacgtgaagaattgcaagaagcattgga

SEQ ID NO: 7 - DNA, 38 bp, synthetic construct
  source 1..38: mol_type = other DNA
  misc_feature 28: note = n is unnatural base, Z
acgtcgattcgccgcgtcgatagacgtncgagaatgcg

SEQ ID NO: 8 - DNA, 38 bp, synthetic construct
  source 1..38: mol_type = other DNA
  misc_feature 6: note = n is unnatural base, P
  misc_feature 11: note = n is unnatural base, P
cgcatnctcgnacgtgaagaattgcaagaagcattgga

SEQ ID NO: 9 - DNA, 38 bp, synthetic construct
  source 1..38: mol_type = other DNA
  misc_feature 28: note = n is unnatural base, Z
  misc_feature 33: note = n is unnatural base, Z
acgtcgattcgccgcgtcgatagacgtncgagnatgcg

SEQ ID NO: 10 - DNA, 38 bp, synthetic construct
  source 1..38: mol_type = other DNA
  misc_feature 5: note = n is unnatural base, P
  misc_feature 10: note = n is unnatural base, P
cgcantctcntacgtgaagaattgcaagaagcattgga

SEQ ID NO: 11 - DNA, 38 bp, synthetic construct
  source 1..38: mol_type = other DNA
  misc_feature 29: note = n is unnatural base, Z
  misc_feature 34: note = n is unnatural base, Z
acgtcgattcgccgcgtcgatagacgtangagantgcg

SEQ ID NO: 12 - DNA, 38 bp, synthetic construct
  source 1..38: mol_type = other DNA
  misc_feature 4: note = n is unnatural base, P
  misc_feature 8: note = n is unnatural base, P
  misc_feature 11: note = n is unnatural base, P
cgcnttcncgnacgtgaagaattgcaagaagcattgga

SEQ ID NO: 13 - DNA, 38 bp, synthetic construct
  source 1..38: mol_type = other DNA
  misc_feature 28: note = n is unnatural base, Z
  misc_feature 31: note = n is unnatural base, Z
  misc_feature 35: note = n is unnatural base, Z
acgtcgattcgccgcgtcgatagacgtncgngaangcg

SEQ ID NO: 14 - DNA, 38 bp, synthetic construct
  source 1..38: mol_type = other DNA
  misc_feature 4: note = n is unnatural base, P
  misc_feature 6: note = n is unnatural base, P
  misc_feature 10: note = n is unnatural base, P
cgcntnctcntacgtgaagaattgcaagaagcattgga

SEQ ID NO: 15 - DNA, 38 bp, synthetic construct
  source 1..38: mol_type = other DNA
  misc_feature 29: note = n is unnatural base, Z
  misc_feature 33: note = n is unnatural base, Z
  misc_feature 35: note = n is unnatural base, Z
acgtcgattcgccgcgtcgatagacgtangagnangcg

SEQ ID NO: 16 - DNA, 38 bp, synthetic construct
  source 1..38: mol_type = other DNA
cgcattctcgtacgtgaagaattgcaagaagcattgga

SEQ ID NO: 17 - DNA, 38 bp, synthetic construct
  source 1..38: mol_type = other DNA
acgtcgattcgccgcgtcgatagacgtacgagaatgcg